European Patent Application EP 4 729 942 A2, published April 22, 2026. Title: METHODS FOR MODULATING HOST CELL SURFACE INTERACTIONS WITH HUMAN CYTOMEGALOVIRUS. Applicant: GENENTECH, INC. The sequence listing filed with the application follows.

SEQUENCE LISTING (8 sequences)

SEQ ID NO: 1 - protein, 741 aa, Human betaherpesvirus 5
MRPGLPSYLIILAVCLFSHLLSSRYGAEAVSEPLDKAFHLLLNTYGRPIRFLRENTTQCTYNSSLRNSTVVRENAISFNFFQSYNQYYVFHMPRCLFAGPLAEQFLNQVDLTETLERYQQRLNTYALVSKDLASYRSFSQQLKAQDSLGEQPTTVPPPIDLSIPHVWMPPQTTPHGWTESHTTSGLHRPHFNQTCILFDGHDLLFSTVTPCLHQGFYLIDELRYVKITLTEDFFVVTVSIDDDTPMLLIFGHLPRVLFKAPYQRDNFILRQTEKHELLVLVKKDQLNRHSYLKDPDFLDAALDFNYLDSALLRNSFHRYAVDVLKSGRCQMLDRRTVEMAFAYALALFAAARQEEAGAQVSVPRALDRQAALLQIQEFMITCLSQTPPRTTLLLYPTAVDLAKRALWTPNQITDITSLVRLVYILSKQNQQHLIPQWALRQIADFALKLHKTHLASFLSAFARQELYLMGSLVHSMLVHTTERREIFIVETGLCSLAELSHFTQLLAHPHHEYLSDLYTPCSSSGRRDHSLERLTRLFPDATVPATVPAALSILSTMQPSTLETFPDLFCLPLGESFSALTVSEHVSYIVTNQYLIKGISYPVSTTVVGQSLIITQTDSQTKCELTRNMHTTHSITVALNISLENCACFQSALLEYDDTQGVINIMYMHDSDDVLFALDPYNEVVVSSPRTHYLMLLKNGTVLEVTDVVVDATDSRLLMMSVYALSAIIGIYLLYRMLKTC

SEQ ID NO: 2 - protein, 279 aa, Human betaherpesvirus 5
MCRRPDCGFSFSPGPVILLWCCLLLPIVSSAAVSVAPTAAEKVPAECPELTRRCLLGEVFEGDKYESWLRPLVNVTGRDGPLSQLIRYRPVTPEAANSVLLDEAFLDTLALLYNNPDQLRALLTLLSSDTAPRWMTVMRGYSECGDGDTPAVYTCVDDLCRGYDLTRLSYGRSIFTEHVLGFELVPPSLFNVVVAIRNEATRTNRAVRLPVSTAAAPEGITLFYGLYNAVKEFCLRHQLDPPLLRHLDKYYAGLPPELKQTRVNLPAHSRYGPQAVDAR

SEQ ID NO: 3 - protein, 171 aa, Human betaherpesvirus 5
MSPKNLTPFLTALWLLLDHSRVPRVRAEECCEFINVNHPPERCYDFKMCNRFTVALRCPDGEVCYSPEKTAEIRGIVTTMTHSLTRQVVHNKLTSCNYNPLYLEADGRIRCGKVNDKAQYLLGAAGSVPYRWINLEYDKITRIVGLNQYLESVKKHKRLDVCRAKMGYMLQ

SEQ ID NO: 4 - protein, 214 aa, Human betaherpesvirus 5
MLRLLLRHHFHCLLLCAVWATPCLASPWSTLTANQNPSPPWSKLTYSKPHDAATFYCPFLYPSPPRSPLQFSGFQRVSTGPECRNETLYLLYNREGQTLVERSSTWVKKVIWYLSGRNQTILQRMPRTASKPSDGNVQISVEDAKIFGAHMVPKQTKLLRFVVNDGTRYQMCVMKLESWAHVFRDYSVSFQVRLTFTEANNQTYTFCTHPNLIV

SEQ ID NO: 5 - protein, 129 aa, Human betaherpesvirus 5
MRLCRVWLSVCLCAVVLGQCQRETAEKNDYYRVPHYWDACSRALPDQTRYKYVEQLVDLTLNYHYDASHGLDNFDVLKRINVTEVSLLISDFRRQNRRGGTNKRTTFNAAGSLAPHARSLEFSVRLFAN

SEQ ID NO: 6 - protein, 591 aa, Homo sapiens
MERGLPLLCAVLALVLAPAGAFRNDKCGDTIKIESPGYLTSPGYPHSYHPSEKCEWLIQAPDPYQRIMINFNPHFDLEDRDCKYDYVEVFDGENENGHFRGKFCGKIAPPPVVSSGPFLFIKFVSDYETHGAGFSIRYEAIFKRGPECSQNYTTPSGVIKSPGFPEKYPNSLECTYIVFVPKMSEIILEFESFDLEPDSNPPGGMFCRYDRLEIWDGFPDVGPHIGRYCGQKTPGRIRSSSGILSMVFYTDSAIAKEGFSANYSVLQSSVSEDFKCMEALGMESGEIHSDQITASSQYSTNWSAERSRLNYPENGWTPGEDSYREWIQVDLGLLRFVTAVGTQGAISKETKKKYYVKTYKIDVSSNGEDWITIKEGNKPVLFQGNTNPTDVVVAVFPKPLITRFVRIKPATWETGISMRFEVYGCKITDYPCSGMLGMVSGLISDSQITSSNQGDRNWMPENIRLVTSRSGWALPPAPHSYINEWLQIDLGEEKIVRGIIIQGGKHRENKVFMRKFKIGYSNNGSDWKMIMDDSKRKAKSFEGNNNYDTPELRTFPALSTRFIRIYPERATHGGLGLRMELLGCEVEAPTA

SEQ ID NO: 7 - protein, 599 aa, Homo sapiens
MDMFPLTWVFLALYFSRHQVRGQPDPPCGGRLNSKDAGYITSPGYPQDYPSHQNCEWIVYAPEPNQKIVLNFNPHFEIEKHDCKYDFIEIRDGDSESADLLGKHCGNIAPPTIISSGSMLYIKFTSDYARQGAGFSLRYEIFKTGSEDCSKNFTSPNGTIESPGFPEKYPHNLDCTFTILAKPKMEIILQFLIFDLEHDPLQVGEGDCKYDWLDIWDGIPHVGPLIGKYCGTKTPSELRSSTGILSLTFHTDMAVAKDGFSARYYLVHQEPLENFQCNVPLGMESGRIANEQISASSTYSDGRWTPQQSRLHGDDNGWTPNLDSNKEYLQVDLRFLTMLTAIATQGAISRETQNGYYVKSYKLEVSTNGEDWMVYRHGKNHKVFQANNDATEVVLNKLHAPLLTRFVRIRPQTWHSGIALRLELFGCRVTDAPCSNMLGMLSGLIADSQISASSTQEYLWSPSAARLVSSRSGWFPRIPQAQPGEEWLQVDLGTPKTVKGVIIQGARGGDSITAVEARAFVRKFKVSYSLNGKDWEYIQDPRTQQPKLFEGNMHYDTPDIRRFDPIPAQYVRVYPERWSPAGIGMRLEVLGCDWTDSKP

SEQ ID NO: 8 - RNA, 20 nt, synthetic construct
  source 1..20: mol_type = other RNA
gggtagtcctgggggtaacc